European Patent Application EP 4 737 482 A1, published May 6, 2026. Title: Humanized anti-MYCT1 antibodies and uses thereof. Applicant: Atheonbio Inc. The sequence listing filed with the application follows.

SEQUENCE LISTING (115 sequences)

SEQ ID NO: 1 - protein, 235 aa, Homo sapiens
MRTQVYEGLCKNYFSLAVLQRDRIKLLFFDILVFLSVFLLFLLFLVDIMANNTTSLGSPWPENFWEDLIMSFTVSMAIGLVLGGFIWAVFICLSRRRRASAPISQWSSSRRSRSSYTHGLNRTGFYRHSGCERRSNLSLASLTFQRQASLEQANSFPRKSSFRASTFHPFLQCPPLPVETESQLVTLPSSNISPTISTSHSLSRPDYWSSNSLRVGLSTPPPPAYESIIKAFPDS

SEQ ID NO: 2 - protein, 19 aa, unidentified
MANNTTSLGSPWPENFWED

SEQ ID NO: 3 - protein, 5 aa, synthetic construct
DYNMH

SEQ ID NO: 4 - protein, 17 aa, synthetic construct
YINPNNGGSSYNRKFKG

SEQ ID NO: 5 - protein, 4 aa, synthetic construct
RFDV

SEQ ID NO: 6 - protein, 16 aa, synthetic construct
KSSQSLLFSDGKTYLN

SEQ ID NO: 7 - protein, 7 aa, synthetic construct
LVSKLDS

SEQ ID NO: 8 - protein, 9 aa, synthetic construct
WQGTHFPQT

SEQ ID NO: 9 - protein, 5 aa, synthetic construct
DFGIH

SEQ ID NO: 10 - protein, 17 aa, synthetic construct
YISSGSRTIHYADTVKG

SEQ ID NO: 11 - protein, 10 aa, synthetic construct
RDWDPEWLAY

SEQ ID NO: 12 - protein, 16 aa, synthetic construct
RSSLSLVHSNGHTYLH

SEQ ID NO: 13 - protein, 7 aa, synthetic construct
KVSNRFS

SEQ ID NO: 14 - protein, 9 aa, synthetic construct
SQSTHVPFT

SEQ ID NO: 15 - protein, 30 aa, synthetic construct
EVQLQQSGPELVKPGASVKMSCKASGYTFT

SEQ ID NO: 16 - protein, 30 aa, synthetic construct
QVQLVQSGAEVKKPGASVKVSCKASGYTFT

SEQ ID NO: 17 - protein, 30 aa, synthetic construct
QVQLVQSGAEVKKPGASVKMSCKASGYTFT

SEQ ID NO: 18 - protein, 14 aa, synthetic construct
WVRQSHGKGLEWIG

SEQ ID NO: 19 - protein, 14 aa, synthetic construct
WVRQAPGQGLEWMG

SEQ ID NO: 20 - protein, 14 aa, synthetic construct
WVRQAPGQGLEWIG

SEQ ID NO: 21 - protein, 32 aa, synthetic construct
KATLTVNKSSRSASMELRSLTSEDSAVYYCAT

SEQ ID NO: 22 - protein, 32 aa, synthetic construct
RVTMTTDTSTSTAYMELRSLRSDDTAVYYCAR

SEQ ID NO: 23 - protein, 32 aa, synthetic construct
RVTMTTDTSTSTAYMELRSLRSDDTAVYYCAT

SEQ ID NO: 24 - protein, 32 aa, synthetic construct
RVTLTTDTSTSTAYMELRSLRSDDTAVYYCAT

SEQ ID NO: 25 - protein, 32 aa, synthetic construct
RVTMTVDTSTSTAYMELRSLRSDDTAVYYCAT

SEQ ID NO: 26 - protein, 32 aa, synthetic construct
RVTMTTDKSTSTAYMELRSLRSDDTAVYYCAT

SEQ ID NO: 27 - protein, 32 aa, synthetic construct
RVTMTVDKSTRTAYMELRSLRSDDTAVYYCAT

SEQ ID NO: 28 - protein, 32 aa, synthetic construct
RVTLTVDKSTRTAYMELRSLRSDDTAVYYCAT

SEQ ID NO: 29 - protein, 11 aa, synthetic construct
WGTGTTVTVSS

SEQ ID NO: 30 - protein, 10 aa, synthetic construct
WGTGTTVTVS

SEQ ID NO: 31 - protein, 11 aa, synthetic construct
WGQGTTVTVSS

SEQ ID NO: 32 - protein, 23 aa, synthetic construct
DVVMTQTPLTLSVTIGHPASISC

SEQ ID NO: 33 - protein, 23 aa, synthetic construct
DVVMTQSPLSLPVTLGQPASISC

SEQ ID NO: 34 - protein, 15 aa, synthetic construct
WLLQRPGQSPKRLIY

SEQ ID NO: 35 - protein, 15 aa, synthetic construct
WFQQRPGQSPRRLIY

SEQ ID NO: 36 - protein, 15 aa, synthetic construct
WLQQRPGQSPRRLIY

SEQ ID NO: 37 - protein, 32 aa, synthetic construct
GVPDRFTGSGSGTDFTLKISRVEAEDLGVYYC

SEQ ID NO: 38 - protein, 32 aa, synthetic construct
GVPDRFSGSGSGTDFTLKISRVEAEDVGVYYC

SEQ ID NO: 39 - protein, 10 aa, synthetic construct
FGGGTKLEIK

SEQ ID NO: 40 - protein, 10 aa, synthetic construct
FGGGTKVEIK

SEQ ID NO: 41 - protein, 113 aa, synthetic construct
EVQLQQSGPELVKPGASVKMSCKASGYTFTDYNMHWVRQSHGKGLEWIGYINPNNGGSSYNRKFKGKATLTVNKSSRSASMELRSLTSEDSAVYYCATRFDVWGTGTTVTVSS

SEQ ID NO: 42 - protein, 112 aa, synthetic construct
DVVMTQTPLTLSVTIGHPASISCKSSQSLLFSDGKTYLNWLLQRPGQSPKRLIYLVSKLDSGVPDRFTGSGSGTDFTLKISRVEAEDLGVYYCWQGTHFPQTFGGGTKLEIK

SEQ ID NO: 43 - protein, 113 aa, synthetic construct
EVQLQQSGPELVKPGASVKMSCKASGYTFTDYNMHWVRQSHGKGLEWIGYINPNQGGSSYNRKFKGKATLTVNKSSRSASMELRSLTSEDSAVYYCATRFDVWGTGTTVTVSS

SEQ ID NO: 44 - protein, 113 aa, synthetic construct
EVQLQQSGPELVKPGASVKMSCKASGYTFTDYNMHWVRQSHGKGLEWIGYINPNSGGSSYNRKFKGKATLTVNKSSRSASMELRSLTSEDSAVYYCATRFDVWGTGTTVTVSS

SEQ ID NO: 45 - protein, 113 aa, synthetic construct
EVQLQQSGPELVKPGASVKMSCKASGYTFTDYNMHWVRQSHGKGLEWIGYINPNNAGSSYNRKFKGKATLTVNKSSRSASMELRSLTSEDSAVYYCATRFDVWGTGTTVTVSS

SEQ ID NO: 46 - protein, 112 aa, synthetic construct
EVQLQQSGPELVKPGASVKMSCKASGYTFTDYNMHWVRQSHGKGLEWIGYINPNNGGSSYNRKFKGKATLTVNKSSRSASMELRSLTSEDSAVYYCATRFDVWGTGTTVTVS

SEQ ID NO: 47 - protein, 113 aa, synthetic construct
QVQLVQSGAEVKKPGASVKVSCKASGYTFTDYNMHWVRQAPGQGLEWMGYINPNNGGSSYNRKFKGRVTMTTDTSTSTAYMELRSLRSDDTAVYYCARRFDVWGQGTTVTVSS

SEQ ID NO: 48 - protein, 113 aa, synthetic construct
QVQLVQSGAEVKKPGASVKVSCKASGYTFTDYNMHWVRQAPGQGLEWMGYINPNNGGSSYNRKFKGRVTMTTDTSTSTAYMELRSLRSDDTAVYYCATRFDVWGQGTTVTVSS

SEQ ID NO: 49 - protein, 113 aa, synthetic construct
QVQLVQSGAEVKKPGASVKVSCKASGYTFTDYNMHWVRQAPGQGLEWMGYINPNNGGSSYNRKFKGRVTLTTDTSTSTAYMELRSLRSDDTAVYYCATRFDVWGQGTTVTVSS

SEQ ID NO: 50 - protein, 113 aa, synthetic construct
QVQLVQSGAEVKKPGASVKVSCKASGYTFTDYNMHWVRQAPGQGLEWMGYINPNNGGSSYNRKFKGRVTMTVDTSTSTAYMELRSLRSDDTAVYYCATRFDVWGQGTTVTVSS

SEQ ID NO: 51 - protein, 113 aa, synthetic construct
QVQLVQSGAEVKKPGASVKVSCKASGYTFTDYNMHWVRQAPGQGLEWMGYINPNNGGSSYNRKFKGRVTMTTDKSTSTAYMELRSLRSDDTAVYYCATRFDVWGQGTTVTVSS

SEQ ID NO: 52 - protein, 113 aa, synthetic construct
QVQLVQSGAEVKKPGASVKVSCKASGYTFTDYNMHWVRQAPGQGLEWMGYINPNNGGSSYNRKFKGRVTMTTDTSTRTAYMELRSLRSDDTAVYYCATRFDVWGQGTTVTVSS

SEQ ID NO: 53 - protein, 113 aa, synthetic construct
QVQLVQSGAEVKKPGASVKMSCKASGYTFTDYNMHWVRQAPGQGLEWMGYINPNNGGSSYNRKFKGRVTMTTDTSTSTAYMELRSLRSDDTAVYYCATRFDVWGQGTTVTVSS

SEQ ID NO: 54 - protein, 113 aa, synthetic construct
QVQLVQSGAEVKKPGASVKVSCKASGYTFTDYNMHWVRQAPGQGLEWIGYINPNNGGSSYNRKFKGRVTMTTDTSTSTAYMELRSLRSDDTAVYYCATRFDVWGQGTTVTVSS

SEQ ID NO: 55 - protein, 113 aa, synthetic construct
QVQLVQSGAEVKKPGASVKVSCKASGYTFTDYNMHWVRQAPGQGLEWMGYINPNNGGSSYNRKFKGRVTMTVDKSTRTAYMELRSLRSDDTAVYYCATRFDVWGQGTTVTVSS

SEQ ID NO: 56 - protein, 113 aa, synthetic construct
QVQLVQSGAEVKKPGASVKVSCKASGYTFTDYNMHWVRQAPGQGLEWMGYINPNNGGSSYNRKFKGRVTLTVDKSTRTAYMELRSLRSDDTAVYYCATRFDVWGQGTTVTVSS

SEQ ID NO: 57 - protein, 113 aa, synthetic construct
QVQLVQSGAEVKKPGASVKMSCKASGYTFTDYNMHWVRQAPGQGLEWMGYINPNNGGSSYNRKFKGRVTLTVDKSTRTAYMELRSLRSDDTAVYYCATRFDVWGQGTTVTVSS

SEQ ID NO: 58 - protein, 113 aa, synthetic construct
QVQLVQSGAEVKKPGASVKMSCKASGYTFTDYNMHWVRQAPGQGLEWIGYINPNNGGSSYNRKFKGRVTLTVDKSTRTAYMELRSLRSDDTAVYYCATRFDVWGQGTTVTVSS

SEQ ID NO: 59 - protein, 113 aa, synthetic construct
QVQLVQSGAEVKKPGASVKVSCKASGYTFTDYNMHWVRQAPGQGLEWMGYINPNSGGSSYNRKFKGRVTMTTDTSTSTAYMELRSLRSDDTAVYYCATRFDVWGQGTTVTVSS

SEQ ID NO: 60 - protein, 113 aa, synthetic construct
QVQLVQSGAEVKKPGASVKVSCKASGYTFTDYNMHWVRQAPGQGLEWIGYINPNSGGSSYNRKFKGRVTMTTDTSTSTAYMELRSLRSDDTAVYYCATRFDVWGQGTTVTVSS

SEQ ID NO: 61 - protein, 112 aa, synthetic construct
DVVMTQTPLTLSVTIGHPASISCKSSQSLLFSEGKTYLNWLLQRPGQSPKRLIYLVSKLDSGVPDRFTGSGSGTDFTLKISRVEAEDLGVYYCWQGTHFPQTFGGGTKLEIK

SEQ ID NO: 62 - protein, 112 aa, synthetic construct
DVVMTQTPLTLSVTIGHPASISCKSSQSLLFSQGKTYLNWLLQRPGQSPKRLIYLVSKLDSGVPDRFTGSGSGTDFTLKISRVEAEDLGVYYCWQGTHFPQTFGGGTKLEIK

SEQ ID NO: 63 - protein, 112 aa, synthetic construct
DVVMTQTPLTLSVTIGHPASISCKSSQSLLFSDAKTYLNWLLQRPGQSPKRLIYLVSKLDSGVPDRFTGSGSGTDFTLKISRVEAEDLGVYYCWQGTHFPQTFGGGTKLEIK

SEQ ID NO: 64 - protein, 112 aa, synthetic construct
DVVMTQSPLSLPVTLGQPASISCKSSQSLLFSDGKTYLNWFQQRPGQSPRRLIYLVSKLDSGVPDRFSGSGSGTDFTLKISRVEAEDVGVYYCWQGTHFPQTFGGGTKVEIK

SEQ ID NO: 65 - protein, 112 aa, synthetic construct
DVVMTQSPLSLPVTLGQPASISCKSSQSLLFSDGKTYLNWLQQRPGQSPRRLIYLVSKLDSGVPDRFSGSGSGTDFTLKISRVEAEDVGVYYCWQGTHFPQTFGGGTKVEIK

SEQ ID NO: 66 - protein, 112 aa, synthetic construct
DVVMTQSPLSLPVTLGQPASISCKSSQSLLFSDAKTYLNWLQQRPGQSPRRLIYLVSKLDSGVPDRFSGSGSGTDFTLKISRVEAEDVGVYYCWQGTHFPQTFGGGTKVEIK

SEQ ID NO: 67 - protein, 30 aa, synthetic construct
EVQLVESGGGLVKPGGSLKLSCAASGFTFS

SEQ ID NO: 68 - protein, 30 aa, synthetic construct
EVQLVESGGGLVKPGGSLRLSCAASGFTFS

SEQ ID NO: 69 - protein, 14 aa, synthetic construct
WVRQAPEKGLEWVG

SEQ ID NO: 70 - protein, 14 aa, synthetic construct
WVRQAPGKGLEWVS

SEQ ID NO: 71 - protein, 14 aa, synthetic construct
WVRQAPGKGLEWVG

SEQ ID NO: 72 - protein, 32 aa, synthetic construct
RFTISRDNAKNTLFLQMTNLRSEDTAIYYCAR

SEQ ID NO: 73 - protein, 32 aa, synthetic construct
RFTISRDNAKNSLYLQMNSLRAEDTAVYYCAR

SEQ ID NO: 74 - protein, 32 aa, synthetic construct
RFTISRDNAKNTLYLQMNSLRAEDTAVYYCAR

SEQ ID NO: 75 - protein, 32 aa, synthetic construct
RFTISRDNAKNSLFLQMNSLRAEDTAVYYCAR

SEQ ID NO: 76 - protein, 32 aa, synthetic construct
RFTISRDNAKNSLYLQMNSLRAEDTAIYYCAR

SEQ ID NO: 77 - protein, 32 aa, synthetic construct
RFTISRDNAKNTLFLQMNSLRAEDTAIYYCAR

SEQ ID NO: 78 - protein, 11 aa, synthetic construct
WGQGTLVTISA

SEQ ID NO: 79 - protein, 11 aa, synthetic construct
WGQGTLVTVSS

SEQ ID NO: 80 - protein, 23 aa, synthetic construct
DVVMTQAPLSLPVSLGDQASISC

SEQ ID NO: 81 - protein, 23 aa, synthetic construct
DIVMTQSPLSLPVTPGEPASISC

SEQ ID NO: 82 - protein, 23 aa, synthetic construct
DVVMTQSPLSLPVTPGEPASISC

SEQ ID NO: 83 - protein, 15 aa, synthetic construct
WYLQKPGQSPKLLIY

SEQ ID NO: 84 - protein, 15 aa, synthetic construct
WYLQKPGQSPQLLIY

SEQ ID NO: 85 - protein, 32 aa, synthetic construct
GVPDRFSGSGSGTDFTLKIRRVEAEDLGVYFC

SEQ ID NO: 86 - protein, 32 aa, synthetic construct; identical to SEQ ID NO: 38

SEQ ID NO: 87 - protein, 32 aa, synthetic construct
GVPDRFSGSGSGTDFTLKIRRVEAEDVGVYYC

SEQ ID NO: 88 - protein, 32 aa, synthetic construct
GVPDRFSGSGSGTDFTLKISRVEAEDVGVYFC

SEQ ID NO: 89 - protein, 32 aa, synthetic construct
GVPDRFSGSGSGTDFTLKIRRVEAEDVGVYFC

SEQ ID NO: 90 - protein, 10 aa, synthetic construct
FGSGTKLEIK

SEQ ID NO: 91 - protein, 10 aa, synthetic construct
FGQGTKLEIK

SEQ ID NO: 92 - protein, 119 aa, synthetic construct
EVQLVESGGGLVKPGGSLKLSCAASGFTFSDFGIHWVRQAPEKGLEWVGYISSGSRTIHYADTVKGRFTISRDNAKNTLFLQMTNLRSEDTAIYYCARRDWDPEWLAYWGQGTLVTISA

SEQ ID NO: 93 - protein, 112 aa, synthetic construct
DVVMTQAPLSLPVSLGDQASISCRSSLSLVHSNGHTYLHWYLQKPGQSPKLLIYKVSNRFSGVPDRFSGSGSGTDFTLKIRRVEAEDLGVYFCSQSTHVPFTFGSGTKLEIK

SEQ ID NO: 94 - protein, 119 aa, synthetic construct
EVQLVESGGGLVKPGGSLRLSCAASGFTFSDFGIHWVRQAPGKGLEWVSYISSGSRTIHYADTVKGRFTISRDNAKNSLYLQMNSLRAEDTAVYYCARRDWDPEWLAYWGQGTLVTVSS

SEQ ID NO: 95 - protein, 119 aa, synthetic construct
EVQLVESGGGLVKPGGSLRLSCAASGFTFSDFGIHWVRQAPGKGLEWVGYISSGSRTIHYADTVKGRFTISRDNAKNSLYLQMNSLRAEDTAVYYCARRDWDPEWLAYWGQGTLVTVSS

SEQ ID NO: 96 - protein, 119 aa, synthetic construct
EVQLVESGGGLVKPGGSLRLSCAASGFTFSDFGIHWVRQAPGKGLEWVSYISSGSRTIHYADTVKGRFTISRDNAKNTLYLQMNSLRAEDTAVYYCARRDWDPEWLAYWGQGTLVTVSS

SEQ ID NO: 97 - protein, 119 aa, synthetic construct
EVQLVESGGGLVKPGGSLRLSCAASGFTFSDFGIHWVRQAPGKGLEWVSYISSGSRTIHYADTVKGRFTISRDNAKNSLFLQMNSLRAEDTAVYYCARRDWDPEWLAYWGQGTLVTVSS

SEQ ID NO: 98 - protein, 119 aa, synthetic construct
EVQLVESGGGLVKPGGSLRLSCAASGFTFSDFGIHWVRQAPGKGLEWVSYISSGSRTIHYADTVKGRFTISRDNAKNSLYLQMNSLRAEDTAIYYCARRDWDPEWLAYWGQGTLVTVSS

SEQ ID NO: 99 - protein, 119 aa, synthetic construct; identical to SEQ ID NO: 94

SEQ ID NO: 100 - protein, 119 aa, synthetic construct
EVQLVESGGGLVKPGGSLRLSCAASGFTFSDFGIHWVRQAPGKGLEWVGYISSGSRTIHYADTVKGRFTISRDNAKNSLYLQMNSLRAEDTAIYYCARRDWDPEWLAYWGQGTLVTVSS

SEQ ID NO: 101 - protein, 119 aa, synthetic construct
EVQLVESGGGLVKPGGSLRLSCAASGFTFSDFGIHWVRQAPGKGLEWVGYISSGSRTIHYADTVKGRFTISRDNAKNTLFLQMNSLRAEDTAIYYCARRDWDPEWLAYWGQGTLVTVSS

SEQ ID NO: 102 - protein, 112 aa, synthetic construct
DVVMTQAPLSLPVSLGDQASISCRSSLSLVHSQGHTYLHWYLQKPGQSPKLLIYKVSNRFSGVPDRFSGSGSGTDFTLKIRRVEAEDLGVYFCSQSTHVPFTFGSGTKLEIK

SEQ ID NO: 103 - protein, 112 aa, synthetic construct
DVVMTQAPLSLPVSLGDQASISCRSSLSLVHSSGHTYLHWYLQKPGQSPKLLIYKVSNRFSGVPDRFSGSGSGTDFTLKIRRVEAEDLGVYFCSQSTHVPFTFGSGTKLEIK

SEQ ID NO: 104 - protein, 112 aa, synthetic construct
DVVMTQAPLSLPVSLGDQASISCRSSLSLVHSNAHTYLHWYLQKPGQSPKLLIYKVSNRFSGVPDRFSGSGSGTDFTLKIRRVEAEDLGVYFCSQSTHVPFTFGSGTKLEIK

SEQ ID NO: 105 - protein, 112 aa, synthetic construct
DIVMTQSPLSLPVTPGEPASISCRSSLSLVHSNGHTYLHWYLQKPGQSPQLLIYKVSNRFSGVPDRFSGSGSGTDFTLKISRVEAEDVGVYYCSQSTHVPFTFGQGTKLEIK

SEQ ID NO: 106 - protein, 112 aa, synthetic construct
DVVMTQSPLSLPVTPGEPASISCRSSLSLVHSNGHTYLHWYLQKPGQSPQLLIYKVSNRFSGVPDRFSGSGSGTDFTLKISRVEAEDVGVYYCSQSTHVPFTFGQGTKLEIK

SEQ ID NO: 107 - protein, 112 aa, synthetic construct
DIVMTQSPLSLPVTPGEPASISCRSSLSLVHSNGHTYLHWYLQKPGQSPKLLIYKVSNRFSGVPDRFSGSGSGTDFTLKISRVEAEDVGVYYCSQSTHVPFTFGQGTKLEIK

SEQ ID NO: 108 - protein, 112 aa, synthetic construct
DIVMTQSPLSLPVTPGEPASISCRSSLSLVHSNGHTYLHWYLQKPGQSPQLLIYKVSNRFSGVPDRFSGSGSGTDFTLKIRRVEAEDVGVYYCSQSTHVPFTFGQGTKLEIK

SEQ ID NO: 109 - protein, 112 aa, synthetic construct
DIVMTQSPLSLPVTPGEPASISCRSSLSLVHSNGHTYLHWYLQKPGQSPQLLIYKVSNRFSGVPDRFSGSGSGTDFTLKISRVEAEDVGVYFCSQSTHVPFTFGQGTKLEIK

SEQ ID NO: 110 - protein, 112 aa, synthetic construct
DVVMTQSPLSLPVTPGEPASISCRSSLSLVHSNGHTYLHWYLQKPGQSPQLLIYKVSNRFSGVPDRFSGSGSGTDFTLKISRVEAEDVGVYFCSQSTHVPFTFGQGTKLEIK

SEQ ID NO: 111 - protein, 112 aa, synthetic construct
DVVMTQSPLSLPVTPGEPASISCRSSLSLVHSNGHTYLHWYLQKPGQSPKLLIYKVSNRFSGVPDRFSGSGSGTDFTLKIRRVEAEDVGVYFCSQSTHVPFTFGQGTKLEIK

SEQ ID NO: 112 - protein, 112 aa, synthetic construct; identical to SEQ ID NO: 93

SEQ ID NO: 113 - protein, 112 aa, synthetic construct
DVVMTQSPLSLPVTPGEPASISCRSSLSLVHSNAHTYLHWYLQKPGQSPQLLIYKVSNRFSGVPDRFSGSGSGTDFTLKISRVEAEDVGVYFCSQSTHVPFTFGQGTKLEIK

SEQ ID NO: 114 - protein, 112 aa, synthetic construct
DVVMTQSPLSLPVTPGEPASISCRSSLSLVHSNAHTYLHWYLQKPGQSPKLLIYKVSNRFSGVPDRFSGSGSGTDFTLKIRRVEAEDVGVYFCSQSTHVPFTFGQGTKLEIK

SEQ ID NO: 115 - protein, 112 aa, synthetic construct
DIVMTQSPLSLPVTPGEPASISCRSSLSLVHSNAHTYLHWYLQKPGQSPKLLIYKVSNRFSGVPDRFSGSGSGTDFTLKISRVEAEDVGVYFCSQSTHVPFTFGQGTKLEIK